European Patent Specification EP 4 301 834 B9, published June 18, 2025. Title: USE OF ENZYMES FOR IMPROVING FRAGRANCE DEPOSITION. Applicant: Novozymes A/S Givaudan SA. The sequence listing filed with the application follows.

SEQUENCE LISTING (8 sequences)

SEQ ID NO: 1 - protein, 524 aa, Paenibacillus polymyxa
VVHGQTAKTITIKVDTFKDRKPISPYIYGTNQDLAGDENMAARRLGGNRMTGYNWENNMSNAGSDWQHSSDNYLCSNGGLTQAECEKPGAVVTSFHDQSLKLGTYSLVTLPMAGYVAADGNGSVQESEAAPSARWNQVVNAKNAPFQLQPDLNDNYVYVDEFVHFLVNKYGTASTKAGVKGYALDNEPALWSHTHPRIHPEKVGAKELVDRSVSLSKAVKAIDAGAEVFGPVLYGFGAYKDLQTAPDWDSVKGNYSWFVDYYLDQMRLSSQVEGKRLLDVFDVHWYPEAMGGGIRITNEVGNDETKKARMQAPRTLWDPTYKEDSWIAQWFSEFLPILPRLKQSVDKYYPGTKLAMTEYSYGGENDISGGIAMTDVLGILGKNDVYMANYWKLKDGVNNYVSAAYKLYRNYDGKNSTFGDTSVSAQTSDIVNSSVHASVTNASDKELHLVVMNKSMDSAFDAQFDLSGAKTYISGKVWGFDKNSSQIKEAAPITQISGNRFTYTVPPLTAYHIVLTTGNDTSPV

SEQ ID NO: 2 - protein, 294 aa, Sordaria fimicola
MRSSTILQTGLVAVLPFAVQAASGSGKSTRYWDCCKPSCAWSGKASVNRPVLACDANNNPLNDANVKSGCDGGSAYTCANNSPWAVNDNLAYGFAATKLSGGTESSWCCACYALTFTSGPVSGKTLVVQSTSTGGDLGSNHFDLNMPGGGVGLFDGCKREFGGLPGAQYGGISSRSECDSFPAALKPGCQWRFDWFKNADNPEFTFKQVQCPSELTSRTGCKRNDDSQFPAFTPPSGGGSNPSTPTTPPSSGGGGSGCAAAMYAQCGGSGFSGCTNCPSGSTCKAINDYYHQCA

SEQ ID NO: 3 - protein, 305 aa, Humicola insolens
MRSSPLLRSAVVAALPVLALAADGRSTRYWDCCKPSCGWAKKAPVNQPVFSCNANFQRITDFDAKSGCEPGGVAYSCADQTPWAVNDDFALGFAATSIAGSNEAGWCCACYELTFTSGPVAGKKMVVQSTSTGGDLGSNHFDLNIPGGGVGIFDGCTPQFGGLPGQRYGGISSRNECDRFPDALKPGCYWRFDWFKNADNPSFSFRQVQCPAELVARTGCRRNDDGNFPAVQIPSSSTSSPVNQPTSTSTTSTSTTSSPPVQPTTPSGCTAERWAQCGGNGWSGCTTCVAGSTCTKINDWYHQCL

SEQ ID NO: 4 - protein, 299 aa, Thielavia terrestris
MRSTPVLRTTLAAALPLVASAASGSGQSTRYWDCCKPSCAWPGKAAVSQPVYACDANFQRLSDFNVQSGCNGGSAYSCADQTPWAVNDNLAYGFAATSIAGGSESSWCCACYALTFTSGPVAGKTMVVQSTSTGGDLGSNHFDIAMPGGGVGIFNGCSSQFGGLPGAQYGGISSRDQCDSFPAPLKPGCQWRFDWFQNADNPTFTFQQVQCPAEIVARSGCKRNDDSSFPVFTPPSGGNGGTGTPTSTAPGSGQTSPGGGSGCTSQKWAQCGGIGFSGCTTCVSGTTCQKLNDYYSQCL

SEQ ID NO: 5 - protein, 295 aa, Staphylotrichum coccosporum
ADGKSTRYWDCCKPSCSWPGKASVNQPVFACSANFQRISDPNVKSGCDGGSAYACADQTPWAVNDNFSYGFAATSISGGNEASWCCGCYELTFTSGPVAGKTMVVQSTSTGGDLGTNHFDLAMPGGGVGIFDGCSPQFGGLAGDRYGGVSSRSQCDSFPAALKPGCYWRFDWFKNADNPTFTFRQVQCPSELVARTGCRRNDDGNFPVFTPPSGGQSSSSSSSSSAKPTSTSTSTTSTKATSTTSTASSQTSSSTGGGCAAQRWAQCGGIGFSGCTTCVSGTTCNKQNDWYSQCL

SEQ ID NO: 6 - protein, 464 aa, Paenibacillus polymyxa
NAGSDWQHSSDNYLCSNGGLTQAECEKPGAVVTSFHDQSLKLGTYSLVTLPMAGYVAADGNGSVQESEAAPSARWNQVVNAKNAPFQLQPDLNDNYVYVDEFVHFLVNKYGTASTKAGVKGYALDNEPALWSHTHPRIHPEKVGAKELVDRSVSLSKAVKAIDAGAEVFGPVLYGFGAYKDLQTAPDWDSVKGNYSWFVDYYLDQMRLSSQVEGKRLLDVFDVHWYPEAMGGGIRITNEVGNDETKKARMQAPRTLWDPTYKEDSWIAQWFSEFLPILPRLKQSVDKYYPGTKLAMTEYSYGGENDISGGIAMTDVLGILGKNDVYMANYWKLKDGVNNYVSAAYKLYRNYDGKNSTFGDTSVSAQTSDIVNSSVHASVTNASDKELHLVVMNKSMDSAFDAQFDLSGAKTYISGKVWGFDKNSSQIKEAAPITQISGNRFTYTVPPLTAYHIVLTTGNDTSPV

SEQ ID NO: 7 - protein, 272 aa, Neurospora tetrasperma
ASGSGQSTRYWDCCKPSCSWSGKASVNRPVLACDANNNPLSDASVKSGCDGGSAYTCANNSPWAVNDQLSYGFAATKLSGGTESSWCCACYALTFTSGPVAGKTMVVQSTSTGGDLGSNHFDINMPGGGVGLFDGCTRQFGGLPGAQYGGISSRSQCDSFPAALKPGCQWRFDWFQNADNPNFTFKQVQCPSELTSRTGCKRNDDSQFPVFTPPSGGGTNPSTPTTPPSSGGGSGCTADKYAQCGGSGWSGCTNCPSGSTCKTINDYYHQCA

SEQ ID NO: 8 - protein, 773 aa, Alkalihalobacillus akibai
AEGNTREDNFKHLLGNDNVKRPSEAGALQLQEVDGQMTLVDQHGEKIQLRGMSTHGLQWFPEILNDNAYKALANDWESNMIRLAMYVGENGYASNPELIKSRVIKGIDLAIENDMYVIVDWHVHAPGDPRDPVYAGAEDFFRDIAALYPNNPHIIYELANEPSSNNNGGAGIPNNEEGWNAVKEYADPIVEMLRDSGNADDNIIIVGSPNWSQRPDLAADNPINDHHTMYTVHFYTGSHAASTESYPPETPNSERGNVMSNTRYALENGVAVFATEWGTSQANGDGGPYFDEADVWIEFLNENNISWANWSLTNKNEVSGAFTPFELGKSNATNLDPGPDHVWAPEELSLSGEYVRARIKGVNYEPIDRTKYTKVLWDFNDGTKQGFGVNSDSPNKELIAVDNENNTLKVSGLDVSNDVSDGNFWANARLSADGWGKSVDILGAEKLTMDVIVDEPTTVAIAAIPQSSKSGWANPERAVRVNAEDFVQQTDGKYKAGLTITGEDAPNLKNIAFHEEDNNMNNIILFVGTDAADVIYLDNIKVIGTEVEIPVVHDPKGEAVLPSVFEDGTRQGWDWAGESGVKTALTIEEANGSNALSWEFGYPEVKPSDNWATAPRLDFWKSDLVRGENDYVAFDFYLDPVRATEGAMNINLVFQPPTNGYWVQAPKTYTINFDELEEANQVNGLYHYEVKINVRDITNIQDDTLLRNMMIIFADVESDFAGRVFVDNVRFEGAATTEPVEPEPVDPGEETPPVDEKEAKKEQKEAEKEEKEE